European Patent Specification EP 3 794 107 B1, published April 29, 2026. Title: METHOD OF CULTURING PROLIFERATIVE HEPATOCYTES. Applicant: INSERM (Institut National de la Santé et de la Recherche Médicale) UNIVERSITÉ DE RENNES 1 ÉCOLE DES HAUTES ÉTUDES EN SANTÉ PUBLIQUE (EHESP) BAFFET Georges LANGOUET Sophie EZAN Frédéric ROSE Sophie CUVELLIER Marie. The sequence listing filed with the application follows.

SEQUENCE LISTING (54 sequences)

SEQ ID NO: 1 - DNA, 20 bp, Artificial Sequence
  primer
gtggacctgacctgccgtct

SEQ ID NO: 2 - DNA, 20 bp, Artificial Sequence
  primer
tgctcttgctgtttcttcgg

SEQ ID NO: 3 - DNA, 20 bp, Artificial Sequence
  primer
gtgcatgaaggacagcctct

SEQ ID NO: 4 - DNA, 22 bp, Artificial Sequence
  primer
ccaaacttttcctccctgaacc

SEQ ID NO: 5 - DNA, 20 bp, Artificial Sequence
  primer
agctggagtctcgcctggaa

SEQ ID NO: 6 - DNA, 19 bp, Artificial Sequence
  primer
gagcctggagaccgagaac

SEQ ID NO: 7 - DNA, 24 bp, Artificial Sequence
  primer
tgcagccaaagtgaagagggaaga

SEQ ID NO: 8 - DNA, 20 bp, Artificial Sequence
  primer
gggcatgtttttgtatgaat

SEQ ID NO: 9 - DNA, 21 bp, Artificial Sequence
  primer
agaatggactggtacctattg

SEQ ID NO: 10 - DNA, 21 bp, Artificial Sequence
  primer
tggagaccttccgacactcct

SEQ ID NO: 11 - DNA, 24 bp, Artificial Sequence
  primer
cttcatccaatggactgcataaat

SEQ ID NO: 12 - DNA, 20 bp, Artificial Sequence
  primer
cctgctcgtggaaatggaga

SEQ ID NO: 13 - DNA, 20 bp, Artificial Sequence
  primer
cgctacttccctgcctttga

SEQ ID NO: 14 - DNA, 21 bp, Artificial Sequence
  primer
tgacgcctcgttgtacatcag

SEQ ID NO: 15 - DNA, 20 bp, Artificial Sequence
  primer
aggaacaaattggacttgga

SEQ ID NO: 16 - DNA, 22 bp, Artificial Sequence
  primer
tgagcaagtttgaaacgcacat

SEQ ID NO: 17 - DNA, 20 bp, Artificial Sequence
  primer
gtccgcagaatggacttgat

SEQ ID NO: 18 - DNA, 20 bp, Artificial Sequence
  primer
taatggaccacatcgctcaa

SEQ ID NO: 19 - DNA, 20 bp, Artificial Sequence
  primer
tgatcagctgcaagaggaga

SEQ ID NO: 20 - DNA, 20 bp, Artificial Sequence
  primer
ccaggacatacacccctttg

SEQ ID NO: 21 - DNA, 20 bp, Artificial Sequence
  primer
cttccaagcggcatagagac

SEQ ID NO: 22 - DNA, 20 bp, Artificial Sequence
  primer
cattcctcttcccctcatca

SEQ ID NO: 23 - DNA, 18 bp, Artificial Sequence
  primer
ccgtccatgcggaagatc

SEQ ID NO: 24 - DNA, 27 bp, Artificial Sequence
  primer
atcattacactaagggccgaagataac

SEQ ID NO: 25 - DNA, 18 bp, Artificial Sequence
  primer
tgagccgcgactgtgatg

SEQ ID NO: 26 - DNA, 20 bp, Artificial Sequence
  primer
catttggtggacccaaagac

SEQ ID NO: 27 - RNA, 20 nt, Artificial Sequence
  primer
cagaaggcaccaacctcaac

SEQ ID NO: 28 - DNA, 20 bp, Artificial Sequence
  primer
ggaggagtgggtgtcgctgt

SEQ ID NO: 29 - DNA, 20 bp, Artificial Sequence
  primer
tgccccattcgttcaagtag

SEQ ID NO: 30 - DNA, 20 bp, Artificial Sequence
  primer
atgccatcttcatccacctt

SEQ ID NO: 31 - DNA, 23 bp, Artificial Sequence
  primer
gtgatgctgagaagtttcgttga

SEQ ID NO: 32 - DNA, 21 bp, Artificial Sequence
  primer
tgtgccttgacctcagcaatg

SEQ ID NO: 33 - DNA, 18 bp, Artificial Sequence
  primer
ttgcgaagatctgagccc

SEQ ID NO: 34 - DNA, 24 bp, Artificial Sequence
  primer
catagcgagcagcccaaagaagaa

SEQ ID NO: 35 - DNA, 20 bp, Artificial Sequence
  primer
cccacttttcctaggtttct

SEQ ID NO: 36 - DNA, 20 bp, Artificial Sequence
  primer
gtaacatactggcagtgttc

SEQ ID NO: 37 - DNA, 20 bp, Artificial Sequence
  primer
cgttgtgtcccttgttgtgc

SEQ ID NO: 38 - DNA, 28 bp, Artificial Sequence
  primer
tcccaagtataacactctacacagacaa

SEQ ID NO: 39 - DNA, 20 bp, Artificial Sequence
  primer
tctctgtccccgcaaagaac

SEQ ID NO: 40 - DNA, 20 bp, Artificial Sequence
  primer
agtcaagctcctcgacgtag

SEQ ID NO: 41 - DNA, 19 bp, Artificial Sequence
  primer
cctccctttggaatggcac

SEQ ID NO: 42 - DNA, 20 bp, Artificial Sequence
  primer
accccggtttcttcttacaa

SEQ ID NO: 43 - DNA, 21 bp, Artificial Sequence
  primer
agctcttctcctgccgtctct

SEQ ID NO: 44 - DNA, 20 bp, Artificial Sequence
  primer
tcaccacttggggatcattt

SEQ ID NO: 45 - DNA, 20 bp, Artificial Sequence
  primer
agcccctgatagagcacaga

SEQ ID NO: 46 - DNA, 20 bp, Artificial Sequence
  primer
aggcctagcaacttcgcata

SEQ ID NO: 47 - DNA, 20 bp, Artificial Sequence
  primer
ctacctgtgatgccgaacaa

SEQ ID NO: 48 - DNA, 20 bp, Artificial Sequence
  primer
agttatcctggcctccgttt

SEQ ID NO: 49 - DNA, 20 bp, Artificial Sequence
  primer
tttaaggtctcggtggagga

SEQ ID NO: 50 - DNA, 20 bp, Artificial Sequence
  primer
gaagacctcctcctcgcact

SEQ ID NO: 51 - DNA, 28 bp, Artificial Sequence
  primer
tcatttcatagtctgaaactttctcctg

SEQ ID NO: 52 - DNA, 23 bp, Artificial Sequence
  primer
gtctcggtgacaaagtcgaagtt

SEQ ID NO: 53 - DNA, 20 bp, Artificial Sequence
  primer
agaagaatcgtcggttgcag

SEQ ID NO: 54 - DNA, 20 bp, Artificial Sequence
  primer
ctcgaggcaccgtagtgttt